European Patent Application EP 4 261 272 A1, published October 18, 2023. Title: MICROORGANISM FOR PRODUCING PANTOIC ACID, AND CONSTRUCTION METHOD THEREFOR AND APPLICATION THEREOF. Applicant: TIANJIN INSTITUTE OF INDUSTRIAL BIOTECHNOLOGY, CHINESE ACADEMY OF SCIENCES. Application EP21932460.5. The sequence listing filed with the application follows.

SEQUENCE LISTING (148 sequences)

SEQ ID NO: 1 - DNA, 1716 bp, Artificial Sequence
  Artificial sequence
atgttgacaaaagcaacaaaagaacaaaaatcccttgtgaaaaacagaggggcggagcttgttgttgattgcttagtggagcaaggtgtcacacatgtatttggcattccaggtgcaaaaattgatgcggtatttgacgctttacaagataaaggacctgaaattatcgttgcccggcacgaacaaaacgcagcattcatggcccaagcagtcggccgtttaactggaaaaccgggagtcgtgttagtcacatcaggaccgggtgcctctaacttggcaacaggcctgctgacagcgaacactgaaggagaccctgtcgttgcgcttgctggaaacgtgatccgtgcagatcgtttaaaacggacacatcaatctttggataatgcggcgctattccagccgattacaaaatacagtgtagaagttcaagatgtaaaaaatataccggaagctgttacaaatgcatttaggatagcgtcagcagggcaggctggggccgcttttgtgagctttccgcaagatgttgtgaatgaagtcacaaatacgaaaaacgtgcgtgctgttgcagcgccaaaactcggtcctgcagcagatgatgcaatcagtgcggccatagcaaaaatccaaacagcaaaacttcctgtcgttttggtcggcatgaaaggcggaagaccggaagcaattaaagcggttcgcaagcttttgaaaaaggttcagcttccatttgttgaaacatatcaagctgccggtaccctttctagagatttagaggatcaatattttggccgtatcggtttgttccgcaaccagcctggcgatttactgctagagcaggcagatgttgttctgacgatcggctatgacccgattgaatatgatccgaaattctggaatatcaatggagaccggacaattatccatttagacgagattatcgctgacattgatcatgcttaccagcctgatcttgaattgatcggtgacattccgtccacgatcaatcatatcgaacacgatgctgtgaaagtggaatttgcagagcgtgagcagaaaatcctttctgatttaaaacaatatatgcatgaaggtgagcaggtgcctgcagattggaaatcagacagagcgcaccctcttgaaatcgttaaagagttgcgtaatgcagtcgatgatcatgttacagtaacttgcgatatcggttcgcacgccatttggatgtcacgttatttccgcagctacgagccgttaacattaatgatcagtaacggtatgcaaacactcggcgttgcgcttccttgggcaatcggcgcttcattggtgaaaccgggagaaaaagtggtttctgtctctggtgacggcggtttcttattctcagcaatggaattagagacagcagttcgactaaaagcaccaattgtacacattgtatggaacgacagcacatatgacatggttgcattccagcaattgaaaaaatataaccgtacatctgcggtcgatttcggaaatatcgatatcgtgaaatatgcggaaagcttcggagcaactggcttgcgcgtagaatcaccagaccagctggcagatgttctgcgtcaaggcatgaacgctgaaggtcctgtcatcatcgatgtcccggttgactacagtgataacattaatttagcaagtgacaagcttccgaaagaattcggggaactcatgaaaacgaaagctctctag

SEQ ID NO: 2 - protein, 571 aa, Artificial sequence
  Artificial sequence
MLTKATKEQKSLVKNRGAELVVDCLVEQGVTHVFGIPGAKIDAVFDALQDKGPEIIVARHEQNAAFMAQAVGRLTGKPGVVLVTSGPGASNLATGLLTANTEGDPVVALAGNVIRADRLKRTHQSLDNAALFQPITKYSVEVQDVKNIPEAVTNAFRIASAGQAGAAFVSFPQDVVNEVTNTKNVRAVAAPKLGPAADDAISAAIAKIQTAKLPVVLVGMKGGRPEAIKAVRKLLKKVQLPFVETYQAAGTLSRDLEDQYFGRIGLFRNQPGDLLLEQADVVLTIGYDPIEYDPKFWNINGDRTIIHLDEIIADIDHAYQPDLELIGDIPSTINHIEHDAVKVEFAEREQKILSDLKQYMHEGEQVPADWKSDRAHPLEIVKELRNAVDDHVTVTCDIGSHAIWMSRYFRSYEPLTLMISNGMQTLGVALPWAIGASLVKPGEKVVSVSGDGGFLFSAMELETAVRLKAPIVHIVWNDSTYDMVAFQQLKKYNRTSAVDFGNIDIVKYAESFGATGLRVESPDQLADVLRQGMNAEGPVIIDVPVDYSDNINLASDKLPKEFGELMKTKAL

SEQ ID NO: 3 - DNA, 88 bp, Artificial sequence
  Artificial sequence
ttatctctggcggtgttgacaagagataacaacgttgatataattgagcccgtattgttagcatgtacgtttaaaccaggaaacagct

SEQ ID NO: 4 - DNA, 492 bp, Artificial sequence
  Artificial sequence
atgcgccggatattatcagtcttactcgaaaatgaatcagacgcgttattccgcgtgattggccttttttcccagcgtggctacaacattgaaagcctgaccgttgcgccaaccgacgatccgacattatcgcgtatgaccatccagaccgtgggcgatgaaaaagtacttgagcagatcgaaaagcaattacacaagctggtcgatgtcttgcgcgtgagtgagttggggcagggcgcgcatgttgagcgggaaatcatgctggtgaaaattcaggccagcggttacgggcgtgacgaagtgaaacgtaatacggaaatattccgtgggcaaattatcgatgtcacaccctcgctttataccgttcaattagcaggcaccagcggtaagcttgatgcatttttagcatcgattcgcgatgtggcgaaaattgtggaggttgctcgctctggtgtggtcggactttcgcgcggcgataaaataatgcgttga

SEQ ID NO: 5 - protein, 163 aa, Artificial sequence
  Artificial sequence
MRRILSVLLENESDALFRVIGLFSQRGYNIESLTVAPTDDPTLSRMTIQTVGDEKVLEQIEKQLHKLVDVLRVSELGQGAHVEREIMLVKIQASGYGRDEVKRNTEIFRGQIIDVTPSLYTVQLAGTSGKLDAFLASIRDVAKIVEVARSGVVGLSRGDKIMR

SEQ ID NO: 6 - DNA, 88 bp, Artificial sequence
  Artificial sequence
ttatctctggcggtgttgacaagagataacaacgttgatataattgagcctctcgccccaccaattcggtttaaaccaggaaacagct

SEQ ID NO: 7 - DNA, 89 bp, Artificial sequence
  Artificial sequence
ttatctctggcggtgttgacaagagataacaacgttgatataattgagcccgtattgttagcatgtacgtttaaaccaggaggtcagca

SEQ ID NO: 8 - DNA, 89 bp, Artificial sequence
  Artificial sequence
ttatctctggcggtgttgacaagagataacaacgttgatataattgagcccgtattgttagcatgtacgtttaaaccaggagggttcga

SEQ ID NO: 9 - DNA, 816 bp, Artificial sequence
  Artificial sequence
atgcccatgtcaggcattgatgcaaagaaaatccgcacccgtcatttccgcgaagctaaagtaaacggccagaaagtttcggttctcaccagctatgatgcgctttcggcgcgcatttttgatgaggctggcgtcgatatgctccttgttggtgattccgctgccaacgttgtgctgggtcgcgataccaccttgtcgatcaccttggatgagatgattgtgctggccaaggcggtgacgatcgctacgaagcgtgcgcttgtggtggttgatctgccgtttggtacctatgaggtgagcccaaatcaggcggtggagtccgcgatccgggtcatgcgtgaaacgggtgcggctgcggtgaagatcgagggtggcgtggagatcgcgcagacgattcgacgcattgttgatgctggaattccggttgtcggccacatcgggtacaccccgcagtccgagcattccttgggcggccacgtggttcagggtcgtggcgcgagttctggaaagctcatcgccgatgcccgcgcgttggagcaggcgggtgcgtttgcggttgtgttggagatggttccagcagaggcagcgcgcgaggttaccgaggatctttccatcaccactatcggaatcggtgccggcaatggcacagatgggcaggttttggtgtggcaggatgccttcggcctcaaccgcggcaagaagccacgcttcgtccgcgagtacgccaccttgggcgattccttgcacgacgccgcgcaggcctacatcgccgatatccacgcgggtaccttcccaggcgaagcggagtccttttaa

SEQ ID NO: 10 - protein, 271 aa, Artificial sequence
  Artificial sequence
MPMSGIDAKKIRTRHFREAKVNGQKVSVLTSYDALSARIFDEAGVDMLLVGDSAANVVLGRDTTLSITLDEMIVLAKAVTIATKRALVVVDLPFGTYEVSPNQAVESAIRVMRETGAAAVKIEGGVEIAQTIRRIVDAGIPVVGHIGYTPQSEHSLGGHVVQGRGASSGKLIADARALEQAGAFAVVLEMVPAEAAREVTEDLSITTIGIGAGNGTDGQVLVWQDAFGLNRGKKPRFVREYATLGDSLHDAAQAYIADIHAGTFPGEAESF

SEQ ID NO: 11 - DNA, 930 bp, Artificial sequence
  Artificial sequence
gtgaccacgaagaaagctgattacatttggttcaatggggagatggttcgctgggaagacgcgaaggtgcatgtgatgtcgcacgcgctgcactatggcacctcggtttttgaaggcatccgttgctacgactcgcacaaaggaccggttgtattccgccatcgtgagcatatgcagcgtctgcatgactccgccaaaatctatcgctttccggtttcgcagagcattgatgagctgatggaagcttgtcgtgacgtgatccgcaaaaacaatctcaccagcgcctatatccgtccgctgatcttcgtcggtgatgttggcatgggcgttaacccgccagcgggatactcaaccgatgtgattatcgccgctttcccgtggggagcgtatctgggcgcagaagcgctggagcaggggatcgatgcgatggtttcctcctggaaccgcgcagcaccaaacaccatcccaaccgcggcaaaagccggtggtaactacctctcttccctgctggtgggtagtgaagcacgccgccacggttatcaggaaggtatcgcgctggatgtgaatggttacatctctgaaggtgcaggcgaaaacctgtttgaagtgaaagacggcgtgctgttcaccccaccgttcacctcctccgcgctgccgggtattacccgtgatgccatcatcaaactggcaaaagagctgggaattgaagtccgtgagcaggtgctgtcgcgcgaatccctgtacctggcggatgaagtgtttatgtccggtactgcggcagaaatcacgccagtgcgcagcgtagatggtattcaggttggtgaaggccgttgcggcccggttaccaaacgcatccagcaagccttcttcggcctcttcactggcgaaaccgaagataaatggggctggttagatcaagttaatcaataa

SEQ ID NO: 12 - protein, 309 aa, Artificial sequence
  Artificial sequence
VTTKKADYIWFNGEMVRWEDAKVHVMSHALHYGTSVFEGIRCYDSHKGPVVFRHREHMQRLHDSAKIYRFPVSQSIDELMEACRDVIRKNNLTSAYIRPLIFVGDVGMGVNPPAGYSTDVIIAAFPWGAYLGAEALEQGIDAMVSSWNRAAPNTIPTAAKAGGNYLSSLLVGSEARRHGYQEGIALDVNGYISEGAGENLFEVKDGVLFTPPFTSSALPGITRDAIIKLAKELGIEVREQVLSRESLYLADEVFMSGTAAEITPVRSVDGIQVGEGRCGPVTKRIQQAFFGLFTGETEDKWGWLDQVNQ

SEQ ID NO: 13 - DNA, 1002 bp, Artificial sequence
  Artificial sequence
atgagccagaatggccgtccggtagtcctcatcgccgataagcttgcgcagtccactgttgacgcgcttggagatgcagtagaagtccgttgggttgacggacctaaccgcccagaactgcttgatgcagttaaggaagcggacgcactgctcgtgcgttctgctaccactgtcgatgctgaagtcatcgccgctgcccctaacttgaagatcgtcggtcgtgccggcgtgggcttggacaacgttgacatccctgctgccactgaagctggcgtcatggttgctaacgcaccgacctctaatattcactccgcttgtgagcacgcaatttctttgctgctgtctactgctcgccagatccctgctgctgatgcgacgctgcgtgagggcgagtggaagcggtcttctttcaacggtgtggaaattttcggaaaaactgtcggtatcgtcggttttggccacattggtcagttgtttgctcagcgtcttgctgcgtttgagaccaccattgttgcttacgatccttacgctaaccctgctcgtgcggctcagctgaacgttgagttggttgagttggatgagctgatgagccgttctgactttgtcaccattcaccttcctaagaccaaggaaactgctggcatgtttgatgcgcagctccttgctaagtccaagaagggccagatcatcatcaacgctgctcgtggtggccttgttgatgagcaggctttggctgatgcgattgagtccggtcacattcgtggcgctggtttcgatgtgtactccaccgagccttgcactgattctcctttgttcaagttgcctcaggttgttgtgactcctcacttgggtgcttctactgaagaggctcaggatcgtgcgggtactgacgttgctgattctgtgctcaaggcgctggctggcgagttcgtggcggatgctgtgaacgtttccggtggtcgcgtgggcgaagaggttgctgtgtggatggatctggcttaa

SEQ ID NO: 14 - protein, 333 aa, Artificial sequence
  Artificial sequence
MSQNGRPVVLIADKLAQSTVDALGDAVEVRWVDGPNRPELLDAVKEADALLVRSATTVDAEVIAAAPNLKIVGRAGVGLDNVDIPAATEAGVMVANAPTSNIHSACEHAISLLLSTARQIPAADATLREGEWKRSSFNGVEIFGKTVGIVGFGHIGQLFAQRLAAFETTIVAYDPYANPARAAQLNVELVELDELMSRSDFVTIHLPKTKETAGMFDAQLLAKSKKGQIIINAARGGLVDEQALADAIESGHIRGAGFDVYSTEPCTDSPLFKLPQVVVTPHLGASTEEAQDRAGTDVADSVLKALAGEFVADAVNVSGGRVGEEVAVWMDLA

SEQ ID NO: 15 - DNA, 2167 bp, Artificial sequence
  Artificial sequence
ttatctctggcggtgttgacaagagataacaacgttgatataattgagcccgtattgttagcatgtacgtttaaaccaggaaacagctatggctcaaatcttcaattttagttctggtccggcaatgctaccggcagaggtgcttaaacaggctcaacaggaactgcgcgactggaacggtcttggtacgtcggtgatggaagtgagtcaccgtggcaaagagttcattcaggttgcagaggaagccgagaaggattttcgcgatcttcttaatgtcccctccaactacaaggtattattctgccatggcggtggtcgcggtcagtttgctgcggtaccgctgaatattctcggtgataaaaccaccgcagattatgttgatgccggttactgggcggcaagtgccattaaagaagcgaaaaaatactgcacgcctaatgtctttgacgccaaagtgactgttgatggtctgcgcgcggttaagccaatgcgtgaatggcaactctctgataatgctgcttatatgcattattgcccgaatgaaaccatcgatggtatcgccatcgacgaaacgccagacttcggcgcagatgtggtggtcgccgctgacttctcttcaaccattctttcccgtccgattgacgtcagccgttatggtgtaatttacgctggcgcgcagaaaaatatcggcccggctggcctgacaatcgtcatcgttcgtgaagatttgctgggcaaagcgaatatcgcgtgtccgtcgattctggattattccatcctcaacgataacggctccatgtttaacacgccgccgacatttgcctggtatctatctggtctggtctttaaatggctgaaagcgaacggcggtgtagctgaaatggataaaatcaatcagcaaaaagcagaactgctatatggggtgattgataacagcgatttctaccgcaatgacgtggcgaaagctaaccgttcgcggatgaacgtgccgttccagttggcggacagtgcgcttgacaaattgttccttgaagagtcttttgctgctggccttcatgcactgaaaggtcaccgtgtggtcggcggaatgcgcgcttctatttataacgccatgccgctggaaggcgttaaagcgctgacagacttcatggttgagttcgaacgccgtcacggttaagtcgacaaaaggagaacaaacatgcctaacattacctggtgcgacctgcctgaagatgtctctttatggccgggtctgcctctttcattaagtggtgatgaagtgatgccactggattaccacgcaggtcgtagcggctggctgctgtatggtcgtgggctggataaacaacgtctgacccaataccagagcaaactgggtgcggcgatggtgattgttgccgcctggtgcgtggaagattatcaggtgattcgtctggcaggttcactcaccgcacgggctacacgcctggcccacgaagcgcagctggatgtcgccccgctggggaaaatcccgcacctgcgcacgccgggtttgctggtgatggatatggactccaccgccatccagattgaatgtattgatgaaattgccaaactggccggaacgggcgagatggtggcggaagtaaccgaacgggcgatgcgcggcgaactcgattttaccgccagcctgcgcagccgtgtggcgacgctgaaaggcgctgacgccaatattctgcaacaggtgcgtgaaaatctgccgctgatgccaggcttaacgcaactggtgctcaagctggaaacgctgggctggaaagtggcgattgcctccggcggctttactttctttgctgaatacctgcgcgacaagctgcgcctgaccgccgtggtagccaatgaactggagatcatggacggtaaatttaccggcaatgtgatcggcgacatcgtagacgcgcagtacaaagcgaaaactctgactcgcctcgcgcaggagtatgaaatcccgctggcgcagaccgtggcgattggcgatggagccaatgacctgccgatgatcaaagcggcagggctggggattgcctaccatgccaagccaaaagtgaatgaaaaggcggaagtcaccatccgtcacgctgacctgatgggggtattctgcatcctctcaggcagcctgaatcagaagtaa

SEQ ID NO: 16 - protein, 362 aa, Artificial sequence
  Artificial sequence
MAQIFNFSSGPAMLPAEVLKQAQQELRDWNGLGTSVMEVSHRGKEFIQVAEEAEKDFRDLLNVPSNYKVLFCHGGGRGQFAAVPLNILGDKTTADYVDAGYWAASAIKEAKKYCTPNVFDAKVTVDGLRAVKPMREWQLSDNAAYMHYCPNETIDGIAIDETPDFGADVVVAADFSSTILSRPIDVSRYGVIYAGAQKNIGPAGLTIVIVREDLLGKANIACPSILDYSILNDNGSMFNTPPTFAWYLSGLVFKWLKANGGVAEMDKINQQKAELLYGVIDNSDFYRNDVAKANRSRMNVPFQLADSALDKLFLEESFAAGLHALKGHRVVGGMRASIYNAMPLEGVKALTDFMVEFERRHG

SEQ ID NO: 17 - protein, 322 aa, Artificial sequence [sequence omitted]

SEQ ID NO: 18 - DNA, 73 bp, Artificial sequence
  Artificial sequence
ccgtgattggtctgctgaccatcctgaacatcgtatacaaactgttttaatgtgacggaagatcacttcgcag

SEQ ID NO: 19 - DNA, 75 bp, Artificial sequence
  Artificial sequence
ataatgttctttgctacaggaaaatcaacaatatgcgcaccagatgccacttatttgttaactgttaattgtcct

SEQ ID NO: 20 - DNA, 72 bp, Artificial sequence
  Artificial sequence
ccgtgattggtctgctgaccatcctgaacatcgtatacaaactgttttaaatgttgacaaaagcaacaaaag

SEQ ID NO: 21 - DNA, 82 bp, Artificial sequence
  Artificial sequence
ataatgttctttgctacaggaaaatcaacaatatgcgcaccagatgccacgcatgagctcctagagagctttcgttttcatg

SEQ ID NO: 22 - DNA, 21 bp, Artificial sequence
  Artificial sequence
tgatgagctacctggtatggc

SEQ ID NO: 23 - DNA, 24 bp, Artificial sequence
  Artificial sequence
cgccgacagagtaataggttttac

SEQ ID NO: 24 - DNA, 75 bp, Artificial sequence
  Artificial sequence
cctctgtttttcacaagggatttttgttcttttgttgcttttgtcaacatttatttgttaactgttaattgtcct

SEQ ID NO: 25 - DNA, 70 bp, Artificial sequence
  Artificial sequence
ccgtgattggtctgctgaccatcctgaacatcgtatacaaactgttttaattatctctggcggtgttgac

SEQ ID NO: 26 - DNA, 70 bp, Artificial sequence
  Artificial sequence
cctctgtttttcacaagggatttttgttcttttgttgcttttgtcaacatagctgtttcctggtttaaac

SEQ ID NO: 27 - DNA, 20 bp, Artificial sequence
  Artificial sequence
gcctgttgccaagttagagg

SEQ ID NO: 28 - DNA, 72 bp, Artificial sequence
  Artificial sequence
ctgacgaaacctcgctccggcggggttttttgttatctgcaattcagtactgtgacggaagatcacttcgca

SEQ ID NO: 29 - DNA, 75 bp, Artificial sequence
  Artificial sequence
tctgcgccggtaaagcgcttacgcgtcgatgttgtgcccgaacttgccatttatttgttaactgttaattgtcct

SEQ ID NO: 30 - DNA, 70 bp, Artificial sequence
  Artificial sequence
ctgacgaaacctcgctccggcggggttttttgttatctgcaattcagtacttatctctggcggtgttgac

SEQ ID NO: 31 - DNA, 70 bp, Artificial sequence
  Artificial sequence
tctgcgccggtaaagcgcttacgcgtcgatgttgtgcccgaacttgccatagctgtttcctggtttaaac

SEQ ID NO: 32 - DNA, 22 bp, Artificial sequence
  Artificial sequence
gttctgcgcggaacacgtatac

SEQ ID NO: 33 - DNA, 20 bp, Artificial sequence
  Artificial sequence
ccgctacaggccatacagac

SEQ ID NO: 34 - DNA, 72 bp, Artificial sequence
  Artificial sequence
tgaactaagaggaagggaacaacattcagaccgaaattgaatttttttcatgtgacggaagatcacttcgca

SEQ ID NO: 35 - DNA, 75 bp, Artificial sequence
  Artificial sequence
ttcacaccctgtgcccgcaacgcatgtaccacccactgtgcgccattcatttatttgttaactgttaattgtcct

SEQ ID NO: 36 - DNA, 70 bp, Artificial sequence
  Artificial sequence
tgaactaagaggaagggaacaacattcagaccgaaattgaatttttttcattatctctggcggtgttgac

SEQ ID NO: 37 - DNA, 71 bp, Artificial sequence
  Artificial sequence
ttcacaccctgtgcccgcaacgcatgtaccacccactgtgcgccattcatagctgtttcctggtttaaacg

SEQ ID NO: 38 - DNA, 22 bp, Artificial sequence
  Artificial sequence
gcataagatatcgctgctgtag

SEQ ID NO: 39 - DNA, 20 bp, Artificial sequence
  Artificial sequence
gccagttttgccagtagcac

SEQ ID NO: 40 - DNA, 72 bp, Artificial sequence
  Artificial sequence
agaacctgattatgcgccggatattatcagtcttactcgaaaatgaatcatgtgacggaagatcacttcgca

SEQ ID NO: 41 - DNA, 75 bp, Artificial sequence
  Artificial sequence
ttcatcgcccacggtctggatggtcatacgcgataatgtcggatcgtcggttatttgttaactgttaattgtcct

SEQ ID NO: 42 - DNA, 74 bp, Artificial sequence
  Artificial sequence
agaacctgattatgcgccggatattatcagtcttactcgaaaatgaatcagacgcgttattccgcgtgattggc

SEQ ID NO: 43 - DNA, 21 bp, Artificial sequence
  Artificial sequence
cacaccagagcgagcaacctc

SEQ ID NO: 44 - DNA, 23 bp, Artificial sequence
  Artificial sequence
atgagctggaaagcaaacttagc

SEQ ID NO: 45 - DNA, 72 bp, Artificial sequence
  Artificial sequence
ataactctaatgtttaaactcttttagtaaatcacagtgagtgtgagcgctgtgacggaagatcacttcgca

SEQ ID NO: 46 - DNA, 75 bp, Artificial sequence
  Artificial sequence
ccgtttatgttgccagacagcgctactgattaagcggattttttcgctttttatttgttaactgttaattgtcct

SEQ ID NO: 47 - DNA, 70 bp, Artificial sequence
  Artificial sequence
ataactctaatgtttaaactcttttagtaaatcacagtgagtgtgagcgcatggctaactacttcaatac

SEQ ID NO: 48 - DNA, 71 bp, Artificial sequence
  Artificial sequence
ccgtttatgttgccagacagcgctactgattaagcggattttttcgctttttaacccgcaacagcaatacg

SEQ ID NO: 49 - DNA, 21 bp, Artificial sequence
  Artificial sequence
catgctaatgtagccaccaaa

SEQ ID NO: 50 - DNA, 20 bp, Artificial sequence
  Artificial sequence
ttgcaccaccatccagataa

SEQ ID NO: 51 - DNA, 75 bp, Artificial sequence
  Artificial sequence
agctgtgccagctgctggcgcagattcagtgtattgaagtagttagccatttatttgttaactgttaattgtcct

SEQ ID NO: 52 - DNA, 70 bp, Artificial sequence
  Artificial sequence
ataactctaatgtttaaactcttttagtaaatcacagtgagtgtgagcgcttatctctggcggtgttgac

SEQ ID NO: 53 - DNA, 72 bp, Artificial sequence
  Artificial sequence
agctgtgccagctgctggcgcagattcagtgtattgaagtagttagccatagctgtttcctggtttaaaccg

SEQ ID NO: 54 - DNA, 20 bp, Artificial sequence
  Artificial sequence
cgcactacatcagagtgctg

SEQ ID NO: 55 - DNA, 73 bp, Artificial sequence
  Artificial sequence
aaacgaccaccattaatggttgtcgaagtacgcagtaaataaaaaatccatgtgacggaagatcacttcgcag

SEQ ID NO: 56 - DNA, 75 bp, Artificial sequence
  Artificial sequence
cggtccgaacggcgcgccagcacgacgaccgtctggggtgttacccgtttttatttgttaactgttaattgtcct

SEQ ID NO: 57 - DNA, 70 bp, Artificial sequence
  Artificial sequence
aaacgaccaccattaatggttgtcgaagtacgcagtaaataaaaaatccaatgcctaagtaccgttccgc

SEQ ID NO: 58 - DNA, 74 bp, Artificial sequence
  Artificial sequence
cggtccgaacggcgcgccagcacgacgaccgtctggggtgttacccgtttttaaccccccagtttcgatttatc

SEQ ID NO: 59 - DNA, 21 bp, Artificial sequence
  Artificial sequence
ctgcggagccgatctctttac

SEQ ID NO: 60 - DNA, 22 bp, Artificial sequence
  Artificial sequence
cgagtaataacgtcctgctgct

SEQ ID NO: 61 - DNA, 75 bp, Artificial sequence
  Artificial sequence
cccgccatattacgaccatgagtggtggtggcggaacggtacttaggcatttatttgttaactgttaattgtcct

SEQ ID NO: 62 - DNA, 70 bp, Artificial sequence
  Artificial sequence
aaacgaccaccattaatggttgtcgaagtacgcagtaaataaaaaatccattatctctggcggtgttgac

SEQ ID NO: 63 - DNA, 78 bp, Artificial sequence
  Artificial sequence
cccgccatattacgaccatgagtggtggtggcggaacggtacttaggcattgctgacctcctggtttaaacgtacatg

SEQ ID NO: 64 - DNA, 20 bp, Artificial sequence
  Artificial sequence
caaccagatcgagcttgatg

SEQ ID NO: 65 - DNA, 20 bp, Artificial sequence
  Artificial sequence
tgcagaaaaccatcgacaag

SEQ ID NO: 66 - DNA, 20 bp, Artificial sequence
  Artificial sequence
caccaatcagcgtgacaact

SEQ ID NO: 67 - DNA, 72 bp, Artificial sequence
  Artificial sequence
gaaggcgaatggctgagatgaaaaacctgaaaattgaggtggtgcgctattgtgacggaagatcacttcgca

SEQ ID NO: 68 - DNA, 75 bp, Artificial sequence
  Artificial sequence
tctcaggctccttaccagtacagggcaacaaacaggattacgatggtggcttatttgttaactgttaattgtcct

SEQ ID NO: 69 - DNA, 70 bp, Artificial sequence
  Artificial sequence
gaaggcgaatggctgagatgaaaaacctgaaaattgaggtggtgcgctatatgaaaccgaccaccatctc

SEQ ID NO: 70 - DNA, 73 bp, Artificial sequence
  Artificial sequence
tctcaggctccttaccagtacagggcaacaaacaggattacgatggtggcttaatggaaactgtgttcttcgc

SEQ ID NO: 71 - DNA, 75 bp, Artificial sequence
  Artificial sequence
tttttttcctgtttgtacttctgcagtaaggagatggtggtcggtttcatttatttgttaactgttaattgtcct

SEQ ID NO: 72 - DNA, 70 bp, Artificial sequence
  Artificial sequence
gaaggcgaatggctgagatgaaaaacctgaaaattgaggtggtgcgctatttatctctggcggtgttgac

SEQ ID NO: 73 - DNA, 70 bp, Artificial sequence
  Artificial sequence
tttttttcctgtttgtacttctgcagtaaggagatggtggtcggtttcatagctgtttcctggtttaaac

SEQ ID NO: 74 - DNA, 20 bp, Artificial sequence
  Artificial sequence
ccaccagcatgacgttaagc

SEQ ID NO: 75 - DNA, 73 bp, Artificial sequence
  Artificial sequence
attatatttgaaattttgtaaaatatttttagtagcttaaatgtgattcatgtgacggaagatcacttcgcag

SEQ ID NO: 76 - DNA, 75 bp, Artificial sequence
  Artificial sequence
aaccagttcgttcgggcaggtttcgcctttttccagagcatgagctcctattatttgttaactgttaattgtcct

SEQ ID NO: 77 - DNA, 70 bp, Artificial sequence
  Artificial sequence
attatatttgaaattttgtaaaatatttttagtagcttaaatgtgattcaatgaaaattaccgtattggg

SEQ ID NO: 78 - DNA, 70 bp, Artificial sequence
  Artificial sequence
aaccagttcgttcgggcaggtttcgcctttttccagagcatgagctcctactaccaggggcgaggcaaac

SEQ ID NO: 79 - DNA, 20 bp, Artificial sequence
  Artificial sequence
gataacggagatcgggaatg

SEQ ID NO: 80 - DNA, 20 bp, Artificial sequence
  Artificial sequence
ctttggctgtcagttcacca

SEQ ID NO: 81 - DNA, 75 bp, Artificial sequence
  Artificial sequence
gtaagccataattgccctaaggcaccgcatcccaatacggtaattttcatttatttgttaactgttaattgtcct

SEQ ID NO: 82 - DNA, 70 bp, Artificial sequence
  Artificial sequence
attatatttgaaattttgtaaaatatttttagtagcttaaatgtgattcattatctctggcggtgttgac

SEQ ID NO: 83 - DNA, 71 bp, Artificial sequence
  Artificial sequence
gtaagccataattgccctaaggcaccgcatcccaatacggtaattttcattcgaaccctcctggtttaaac

SEQ ID NO: 84 - DNA, 20 bp, Artificial sequence
  Artificial sequence
cttttgacggcatcggaaac

SEQ ID NO: 85 - DNA, 73 bp, Artificial sequence
  Artificial sequence
gtaggaaagttaactacggatgtacattatggaactgacgactcgcactttgtgacggaagatcacttcgcag

SEQ ID NO: 86 - DNA, 75 bp, Artificial sequence
  Artificial sequence
gcgtttgccacctgtgcaatattacttcagacggtccgcgagataacgctttatttgttaactgttaattgtcct

SEQ ID NO: 87 - DNA, 20 bp, Artificial sequence
  Artificial sequence
cagctcatcaaccaggtcaa

SEQ ID NO: 88 - DNA, 20 bp, Artificial sequence
  Artificial sequence
aaaagccgtcacgttattgg

SEQ ID NO: 89 - DNA, 71 bp, Artificial sequence
  Artificial sequence
gtaggaaagttaactacggatgtacattatggaactgacgactcgcacttatgttaaagcgtgaaatgaac

SEQ ID NO: 90 - DNA, 70 bp, Artificial sequence
  Artificial sequence
gcgtttgccacctgtgcaatattacttcagacggtccgcgagataacgctttatgcgtaaaccgggtaac

SEQ ID NO: 91 - DNA, 75 bp, Artificial sequence
  Artificial sequence
tgccacagttcggcatcataatcggcaatgttcatttcacgctttaacatttatttgttaactgttaattgtcct

SEQ ID NO: 92 - DNA, 70 bp, Artificial sequence
  Artificial sequence
gtaggaaagttaactacggatgtacattatggaactgacgactcgcacttttatctctggcggtgttgac

SEQ ID NO: 93 - DNA, 70 bp, Artificial sequence
  Artificial sequence
tgccacagttcggcatcataatcggcaatgttcatttcacgctttaacatagctgtttcctggtttaaac

SEQ ID NO: 94 - DNA, 20 bp, Artificial sequence
  Artificial sequence
ccaggttcatacccagaacg

SEQ ID NO: 95 - DNA, 72 bp, Artificial sequence
  Artificial sequence
ttgatttagtgttttttgacatttttttagctcttaatattgtcttattctgtgacggaagatcacttcgca

SEQ ID NO: 96 - DNA, 75 bp, Artificial sequence
  Artificial sequence
cgagcgccgcaaagcgtgtgttgttcgtacaaaggagtctgttgtgccatttatttgttaactgttaattgtcct

SEQ ID NO: 97 - DNA, 70 bp, Artificial sequence
  Artificial sequence
ttgatttagtgttttttgacatttttttagctcttaatattgtcttattcttatctctggcggtgttgac

SEQ ID NO: 98 - DNA, 71 bp, Artificial sequence
  Artificial sequence
cgagcgccgcaaagcgtgtgttgttcgtacaaaggagtctgttgtgccatagctgtttcctggtttaaacg

SEQ ID NO: 99 - DNA, 20 bp, Artificial sequence
  Artificial sequence
ccaggcaatgggattaaacg

SEQ ID NO: 100 - DNA, 20 bp, Artificial sequence
  Artificial sequence
gtggcggagttaacaacgag

SEQ ID NO: 101 - DNA, 72 bp, Artificial sequence
  Artificial sequence
aatcactgctggatgcgaccgcatacgaagcattgttagaagacgagtaatgtgacggaagatcacttcgca

SEQ ID NO: 102 - DNA, 75 bp, Artificial sequence
  Artificial sequence
cgttcaataaaagcgccgctgttttcaagctggcttaacgtctgtgtcatttatttgttaactgttaattgtcct

SEQ ID NO: 103 - DNA, 70 bp, Artificial sequence
  Artificial sequence
aatcactgctggatgcgaccgcatacgaagcattgttagaagacgagtaattatctctggcggtgttgac

SEQ ID NO: 104 - DNA, 71 bp, Artificial sequence
  Artificial sequence
cgttcaataaaagcgccgctgttttcaagctggcttaacgtctgtgtcatagctgtttcctggtttaaacg

SEQ ID NO: 105 - DNA, 22 bp, Artificial sequence
  Artificial sequence
atgagcaacgtaccagcagaac

SEQ ID NO: 106 - DNA, 21 bp, Artificial sequence
  Artificial sequence
gaagttgagcagtgcttcaag

SEQ ID NO: 107 - DNA, 73 bp, Artificial sequence
  Artificial sequence
aggtacttccatgtcgagtaagttagtactggttctgaactgcggtagtttgtgacggaagatcacttcgcag

SEQ ID NO: 108 - DNA, 75 bp, Artificial sequence
  Artificial sequence
ggtcggcagaacgctgtaccgctttgtaggtggtgttaccggtgttcagattatttgttaactgttaattgtcct

SEQ ID NO: 109 - DNA, 72 bp, Artificial sequence
  Artificial sequence
aggtacttccatgtcgagtaagttagtactggttctgaactgcggtagttatgcccatgtcaggcattgatg

SEQ ID NO: 110 - DNA, 70 bp, Artificial sequence
  Artificial sequence
ggtcggcagaacgctgtaccgctttgtaggtggtgttaccggtgttcagattaaaaggactccgcttcgc

SEQ ID NO: 111 - DNA, 20 bp, Artificial sequence
  Artificial sequence
cgggacaacgttcaaaacat

SEQ ID NO: 112 - DNA, 20 bp, Artificial sequence
  Artificial sequence
attgcccatcttcttgttgg

SEQ ID NO: 113 - DNA, 70 bp, Artificial sequence
  Artificial sequence
aggtacttccatgtcgagtaagttagtactggttctgaactgcggtagttttatctctggcggtgttgac

SEQ ID NO: 114 - DNA, 70 bp, Artificial sequence
  Artificial sequence
cggaaatgacgggtgcggattttctttgcatcaatgcctgacatgggcatagctgtttcctggtttaaac

SEQ ID NO: 115 - DNA, 75 bp, Artificial sequence
  Artificial sequence
cggaaatgacgggtgcggattttctttgcatcaatgcctgacatgggcatttatttgttaactgttaattgtcct

SEQ ID NO: 116 - DNA, 20 bp, Artificial sequence
  Artificial sequence
accggaattccagcatcaac

SEQ ID NO: 117 - DNA, 72 bp, Artificial sequence
  Artificial sequence
cacaaccacatcacaacaaatccgcgcctgagcgcaaaaggaatataaaatgtgacggaagatcacttcgca

SEQ ID NO: 118 - DNA, 75 bp, Artificial sequence
  Artificial sequence
cgaaccatctccccattgaaccaaatgtaatcagctttcttcgtggtcatttatttgttaactgttaattgtcct

SEQ ID NO: 119 - DNA, 74 bp, Artificial sequence
  Artificial sequence
cacaaccacatcacaacaaatccgcgcctgagcgcaaaaggaatataaaagtgaccacgaagaaagctgattac

SEQ ID NO: 120 - DNA, 27 bp, Artificial sequence
  Artificial sequence
ttattgattaacttgatctaaccagcc

SEQ ID NO: 121 - DNA, 22 bp, Artificial sequence
  Artificial sequence
atgatgcaacatcaggtcaatg

SEQ ID NO: 122 - DNA, 72 bp, Artificial sequence
  Artificial sequence
gccgaaaacccgaacgcgatgttcgtattgtggaaagaccacactgcggttgtgacggaagatcacttcgca

SEQ ID NO: 123 - DNA, 75 bp, Artificial sequence
  Artificial sequence
tcacgcatgttatcgccaaaacggcagactttcagatgacgggtatcctgttatttgttaactgttaattgtcct

SEQ ID NO: 124 - DNA, 70 bp, Artificial sequence
  Artificial sequence
gccgaaaacccgaacgcgatgttcgtattgtggaaagaccacactgcggtatgagccagaatggccgtcc

SEQ ID NO: 125 - DNA, 71 bp, Artificial sequence
  Artificial sequence
tcacgcatgttatcgccaaaacggcagactttcagatgacgggtatcctgttaagccagatccatccacac

SEQ ID NO: 126 - DNA, 20 bp, Artificial sequence
  Artificial sequence
caccagcgtagagtggtatc

SEQ ID NO: 127 - DNA, 21 bp, Artificial sequence
  Artificial sequence
ctgcagaccggttgacatcac

SEQ ID NO: 128 - DNA, 75 bp, Artificial sequence
  Artificial sequence
tgcgcaagcttatcggcgatgaggactaccggacggccattctggctcatttatttgttaactgttaattgtcct

SEQ ID NO: 129 - DNA, 70 bp, Artificial sequence
  Artificial sequence
gccgaaaacccgaacgcgatgttcgtattgtggaaagaccacactgcggtttatctctggcggtgttgac

SEQ ID NO: 130 - DNA, 70 bp, Artificial sequence
  Artificial sequence
tgcgcaagcttatcggcgatgaggactaccggacggccattctggctcatagctgtttcctggtttaaac

SEQ ID NO: 131 - DNA, 20 bp, Artificial sequence
  Artificial sequence
tctggcgagcagtagacagc

SEQ ID NO: 132 - DNA, 72 bp, Artificial sequence
  Artificial sequence
atgacattctccctttttggtgacaaatttacccgccactccggcattactgtgacggaagatcacttcgca

SEQ ID NO: 133 - DNA, 75 bp, Artificial sequence
  Artificial sequence
ttagtgactttcagcccaggctctttctatctcttccgccagaatcttcattatttgttaactgttaattgtcct

SEQ ID NO: 134 - DNA, 64 bp, Artificial sequence
  Artificial sequence
gcaccaggtaatgttaggcatgtttgttctccttttgtcgacttaaccgtgacggcgttcgaac

SEQ ID NO: 135 - DNA, 64 bp, Artificial sequence
  Artificial sequence
gttcgaacgccgtcacggttaagtcgacaaaaggagaacaaacatgcctaacattacctggtgc

SEQ ID NO: 136 - DNA, 73 bp, Artificial sequence
  Artificial sequence
gatatcccgctatgacattctccctttttggtgacaaatttacccgccacatggctcaaatcttcaattttag

SEQ ID NO: 137 - DNA, 73 bp, Artificial sequence
  Artificial sequence
ttagtgactttcagcccaggctctttctatctcttccgccagaatcttcattacttctgattcaggctgcctg

SEQ ID NO: 138 - DNA, 21 bp, Artificial sequence
  Artificial sequence
gttcggatatgaactggcagg

SEQ ID NO: 139 - DNA, 20 bp, Artificial sequence
  Artificial sequence
caaacacgttgcattggctg

SEQ ID NO: 140 - DNA, 75 bp, Artificial sequence
  Artificial sequence
tctgccggtagcattgccggaccagaactaaaattgaagatttgagccatttatttgttaactgttaattgtcct

SEQ ID NO: 141 - DNA, 20 bp, Artificial sequence
  Artificial sequence
cagagagttgccattcacgc

SEQ ID NO: 142 - DNA, 70 bp, Artificial sequence
  Artificial sequence
gatatcccgctatgacattctccctttttggtgacaaatttacccgccacttatctctggcggtgttgac

SEQ ID NO: 143 - DNA, 70 bp, Artificial sequence
  Artificial sequence
tctgccggtagcattgccggaccagaactaaaattgaagatttgagccatagctgtttcctggtttaaac

SEQ ID NO: 144 - DNA, 72 bp, Artificial sequence
  Artificial sequence
tgttattagttcgttactggaagtccagtcaccttgtcaggagtattatctgtgacggaagatcacttcgca

SEQ ID NO: 145 - DNA, 75 bp, Artificial sequence
  Artificial sequence
aaagcgggtataaattcgcccatccgttgcagatgggcgagtaagaagtattatttgttaactgttaattgtcct

SEQ ID NO: 146 - DNA, 70 bp, Artificial sequence
  Artificial sequence
aagcgggtataaattcgcccatccgttgcagatgggcgagtaagaagtagataatactcctgacaaggtg

SEQ ID NO: 147 - DNA, 20 bp, Artificial sequence
  Artificial sequence
ccagtgaagatgaagtctcg

SEQ ID NO: 148 - DNA, 20 bp, Artificial sequence
  Artificial sequence
atggatcgcacagtttggag